European Patent Application EP 4 726 040 A1, published April 15, 2026. Title: Psychrophilic and thermolabile CRISPR ribonucleoprotein complex and the use thereof. Applicant: Consejo Superior de Investigaciones Cientificas (CSIC). Application EP. The sequence listing filed with the application follows.

SEQUENCE LISTING (30 sequences)

SEQ ID NO: 1 - protein, 991 aa, unidentified
MTKKVLSIDPGVTSIGWTLTEQNEKGHLTKFIDGGSRIFNSVKEAKSGTFKNEKRRAKRTTRRNKYRSNRRMAKLENYLIKNDFLSNKISSLSDHTGLVQQIIGNPYHLRKKALYEPLTNEELAWAIIHLAKRRGFLSSSKSLTPEEKKEQARADELATLMKKEKCKTLGEYFSNLYDKGEKIRGEKLKRQLIQDELELILNKQMETNSLITYKFVNDINTIIFNQRPLKTQKRISLCKFESFGKIKKHTAAKLHPLSQQFILWGFINNLKYNDNSGGMQELTLEQKNVVFDLLWTNKEVTFKKIIKELKLTPETTFNFQKGEDDKVKGNQLLNYFKAKTKTWFNSLSEQQKIDLIQDLSTINDLTGFALKKRIYNHWTKDEEIIENLLLTSDKLPQGYTSLSLKATKKILPFLKAGNKYYEAEKKAYPNFTINTKKVNKLPPVEGISNTVVLKSCSQVRHLVNAIVDKYGEIDIIKIELARDLSKSKKQISETNILNSKNKSLNDEAISYLHKNNIDVNHDNITKYKLWKESESSDKQHRSCYPEQDSDGNWFFPTINLNDLYGANAIYEIEHIIPKSISGDDSFANKALCKHKTNAQKGNKTPYDYYFQKGGQELIDMIAKTAYSQFGKWKGKKFVTSTEKYLDENDIQKRYLNDTRYLAVFLKEYLQPVCKDKIVVSKGGFTAIIRQSLNLNILLGNEFNKNRGDYRHHMVDAFCTSLISPKVLDIINIMRKQFNKKTEKYKECETKLNDYIKNVKNDFIKHFDNVITSHEVESKLKGELEEETLYGHEKIKLDDGSIITKLFQHKPYEEVISKYNSPEEVLKAHDNLEISLPKGLKKYLENNNKLPDMFQGWKRIKKYYNNIDENNFNINIYRAIHNEKEKVIAYKKTQENAYIIVYNDFKNETISKMNEISNKPKFNNVFCKLYKGDLIQDSENNIYKIYQLLSDKRIALHPVNIQPIKTKRKSVKLIFDKEKMYKIKVNILGHII

SEQ ID NO: 2 - DNA, 2973 bp, unidentified
  source 1..2973: mol_type = genomic DNA
atgacaaaaaaagtattatcaatagaccctggcgttacctctatcggatggacattaacagaacaaaatgaaaaaggacacttaactaaattcattgatggcggttcaagaattttcaactctgtaaaagaagctaaaagtggtacatttaaaaatgaaaaaagaagagctaaaagaacaaccagaaggaataaatacagatctaatcgaagaatggctaagttagaaaactatttaattaaaaatgacttcttatctaacaaaataagctctctttctgatcatactggacttgttcaacaaattataggtaatccttaccatttaagaaaaaaagcactttacgaaccattaactaacgaagaattagcttgggctattattcatttagcaaaaagaagaggtttcttatcaagctctaaatcattaacaccagaagaaaagaaagaacaggcaagagccgatgaattagctactcttatgaaaaaagaaaaatgtaaaacacttggtgaatacttttctaatctatatgataaaggtgaaaaaatacgtggtgaaaaattaaaaagacaacttattcaagatgaattagaattaatcttaaataaacaaatggaaactaattctttaattacttataaatttgttaatgatattaatactattatttttaatcaaagaccacttaaaactcaaaaaagaatttctctatgtaaatttgaatcttttggtaaaataaaaaaacatactgcggctaaacttcatcctttaagtcaacaatttattctttggggatttattaataatttaaaatataatgataactctggcggcatgcaagaattaacattagaacaaaaaaatgttgtctttgatttattgtggacaaataaagaagttacctttaaaaaaattattaaagaactaaaattaacgcctgaaactacttttaattttcaaaaaggtgaagatgataaagtaaaagggaatcaattactcaattactttaaagctaaaacaaaaacatggtttaattcattatcagaacaacaaaaaattgatttaatacaagacctatcaactataaatgatttaacaggttttgctcttaaaaagagaatttataatcattggacaaaagatgaagaaattattgaaaatctattattaacttctgataaactaccacaaggttatacttccttatcgcttaaagcgacaaaaaaaatattaccatttttaaaagcaggtaataaatactatgaagcagagaaaaaagcataccctaacttcacaattaatactaagaaagttaataaacttccaccagttgagggtataagcaatacagttgtattaaaatcttgctcacaagtaagacaccttgttaatgctattgttgataaatatggtgaaattgatattattaaaattgaattagcaagagatttatcaaaaagtaaaaaacaaatttctgaaactaatattttaaatagcaaaaataaatcattaaatgatgaagctatctcatatttacataaaaataatattgacgttaatcatgacaacattactaaatacaaactatggaaagaaagcgaaagtagtgataaacaacatcgttcttgttatccagaacaagatagtgatggtaactggttctttcctactattaatttaaatgacttgtatggtgctaacgccatttatgaaatagaacatattattcctaaatcaatatcaggtgatgattcatttgcaaacaaagctttatgtaaacataaaacaaatgctcaaaaaggtaataaaacaccttatgattactattttcaaaaaggtggtcaagaacttatagatatgatagcaaaaacagcttattctcaatttggtaaatggaaaggtaaaaagtttgtaacatctactgaaaaatatttagatgaaaatgatattcaaaaacgatacttaaatgatactcgctatttagctgtatttttaaaagaatatcttcaacctgtttgtaaagataaaattgttgtttcaaaaggtggatttaccgctattattagacaatctttaaatcttaatattttattaggcaatgaatttaataaaaatcgtggtgattatagacatcatatggttgatgctttttgtacaagtctaatttctccaaaagttttagatattattaatattatgagaaaacaatttaataagaaaactgaaaaatataaagagtgtgaaactaaattaaatgattatattaaaaatgttaaaaatgattttattaaacactttgataatgttattacttctcatgaagttgaaagcaaattaaaaggtgaattagaagaagaaactctatatggtcatgaaaaaattaaattagacgatggatctattattacaaaactttttcaacataaaccttatgaagaagttatttcaaaatacaatagtccagaagaagtactaaaagctcatgataatttagaaattagtttaccaaaaggtctaaaaaaatatttagaaaacaataataaactacctgatatgtttcaagggtggaagcgtataaaaaaatattataacaatattgatgaaaataattttaatattaatatatatagagctattcataatgaaaaagaaaaagttattgcttataaaaaaacgcaggaaaatgcttacattattgtttacaatgattttaaaaatgaaaccattagtaaaatgaatgaaatatctaataaacctaaatttaataatgtattttgcaaattatataaaggagatttaatccaagattctgaaaataatatatataaaatttatcaacttttaagtgataaaagaatagctttacatcctgttaatattcaacctataaaaactaaaagaaaatctgtaaaattaatttttgataaagaaaaaatgtataaaataaaagtaaatattttaggtcatattatt

SEQ ID NO: 3 - RNA, 36 nt, unidentified
  source 1..36: mol_type = other RNA
attgtaattagttaacatttattatatacttaaaat

SEQ ID NO: 4 - RNA, 111 nt, unidentified
  source 1..111: mol_type = other RNA; note = antisense_RNA
tttcttttttcggataactttagctcaaagttatctgataaatatcaaattttgaatgctgttgttacaacagaataacattatgtgatcaattgtaaataatatatgaat

SEQ ID NO: 5 - RNA, 115 nt, unidentified
  source 1..115: mol_type = other RNA
attgtaattagttaacgaaagttaactagtgtattacaataagacaacattgttgtcgtaagttttaaactataaatagtctattgaaactcgatttcaataggcttttttcttt

SEQ ID NO: 6 - DNA, 20 bp, Homo sapiens
  source 1..20: mol_type = other DNA
tgctgacgtaggtagtgctt

SEQ ID NO: 7 - DNA, 20 bp, Homo sapiens
  source 1..20: mol_type = other DNA
cccggaactggaccccgccc

SEQ ID NO: 8 - DNA, 20 bp, Homo sapiens
  source 1..20: mol_type = other DNA
agctggaggaggaagggcct

SEQ ID NO: 9 - DNA, 20 bp, Homo sapiens
  source 1..20: mol_type = genomic DNA
gagccgtggtccgcgcgggg

SEQ ID NO: 10 - DNA, 20 bp, Homo sapiens
  source 1..20: mol_type = other DNA
tggacgaaaagtttcagtgc

SEQ ID NO: 11 - DNA, 399 bp, synthetic construct
  source 1..399: mol_type = other DNA
aaggtcgggcaggaagagggcctatttcccatgattccttcatatttgcatatacgatacaaggctgttagagagataattagaattaatttgactgtaaacacaaagatattagtacaaaatacgtgacgtagaaagtaataatttcttgggtagtttgcagttttaaaattatgttttaaaatggactatcatatgcttaccgtaacttgaaagtatttcgatttcttggctttatatatcttgtggaaaggacgaaacaccgagccgtggtccgcgcggggattgtaattagttaacgaaagttaactagtgtattacaataagacaacattgttgtcgtaagttttaaactataaatagtctattgaaactcgatttcaataggcttttttcttt

SEQ ID NO: 12 - DNA, 399 bp, synthetic construct
  source 1..399: mol_type = other DNA
aaggtcgggcaggaagagggcctatttcccatgattccttcatatttgcatatcgatacaaggctgttagagagataattagaattaatttgactgtaaacacaaagatattagtacaaaatacgtgacgtagaaagtaataatttcttgggtagtttgcagttttaaaattatgttttaaaatggactatcatatgcttaccgtaacttgaaagtatttcgatttcttggctttatatatcttgtggaaaggacgaaacacctggacgaaaagtttcagtgcattgtaattagttaacgaaagttaactagtgtattacaataagacaacattgttgtcgtaagttttaaactataaatagtctattgaaactcgatttcaataggcttttttctttt

SEQ ID NO: 13 - RNA, 20 nt, synthetic construct
  source 1..20: mol_type = other RNA
gagccgtggtccgcgcgggg

SEQ ID NO: 14 - RNA, 20 nt, synthetic construct
  source 1..20: mol_type = other RNA
tggacgaaaagtttcagtgc

SEQ ID NO: 15 - DNA, 2970 bp, synthetic construct
  source 1..2970: mol_type = other DNA
accaagaaagtgctgagcatcgaccctggcgtgaccagcatcggctggaccctgaccgagcagaacgagaagggccatctcacaaagtttatcgacggcggcagcagaatcttcaactccgtgaaggaagccaagtctggtacatttaagaacgagaaacggcgggcaaagcgaacaacaagaaggaacaagtacagaagcaatagaagaatggccaaactggaaaactacctgatcaagaacgattttctgtctaacaagatctccagcctgtcagaccacacaggcctggtccagcagatcattggaaatccttatcacctgagaaagaaagctctgtacgagcctctgaccaacgaggaattggcctgggccatcatccacctggctaaaagaagaggcttcctgagcagctctaaaagcctgaccccagaagaaaagaaagaacaggccagagcagatgagctggccaccctcatgaagaaagagaagtgcaagaccctgggagaatacttcagcaatctgtatgataagggcgaaaagatcagaggcgaaaagctgaaaagacagctgatccaggacgagctggagctgatcctgaacaagcagatggaaaccaacagcctgatcacctacaagttcgtgaacgatatcaacaccattatcttcaaccagagacctctgaaaacccagaaaagaatctctctgtgtaaattcgagtcttttggcaagatcaagaaacacaccgccgccaagctgcatcctctgagccagcaatttatactctggggcttcatcaacaacctgaagtacaatgacaacagcggcggcatgcaggagctgaccctggaacaaaagaacgtggtgttcgacctgctgtggacgaacaaggaagtgacctttaagaagattatcaaagagctgaagctgacccctgagaccaccttcaactttcagaagggcgaggacgacaaggtgaagggcaaccagctgctgaactacttcaaggccaagaccaagacatggttcaacagcctgtctgagcagcagaagatcgacctcatccaggacctgtctaccatcaatgatctaaccggcttcgccctgaagaagcggatctacaaccactggaccaaggacgaggaaatcattgagaatctgctgctgacatccgacaaactgcctcagggctacaccagcctgtcgctgaaggccacaaagaagatcctgcccttcctgaaggccggcaacaaatactacgaggccgagaagaaggcctaccccaacttcaccatcaacacgaaaaaagtgaacaagctcccacctgtggaaggcatcagtaataccgtggtgctgaagtcctgtagccaagtgcggcacctggtgaacgccatcgttgacaagtatggcgagatcgacatcatcaagatcgagctggcccgggatctctccaagagcaagaagcagatctccgaaaccaacatcctgaactctaagaataaaagcctgaatgacgaagctatctcatatctgcataagaacaacatcgatgtgaatcacgataatatcaccaaatacaaactgtggaaggaatctgaatccagcgataaacagcacagatcttgttaccctgagcaagatagcgacggcaattggttcttccctacaatcaacctgaatgacctgtacggcgccaacgctatctacgagatcgagcacatcatccctaagagcatcagcggcgacgacagcttcgccaataaggccctgtgcaaacacaaaaccaacgcccagaaaggcaacaaaacaccctacgactactacttccaaaaaggaggacaggagctgattgacatgatcgcgaagacagcctacagccagttcggcaagtggaagggaaagaagttcgtgacaagcaccgagaagtacctggacgagaacgacatccaaaagagatacctgaacgacaccagatacctggccgtgttcctgaaggagtacctgcagcccgtgtgcaaggacaaaatcgtggtcagcaagggcggattcaccgccatcattcggcagagccttaacctgaacatcctgctgggaaatgagttcaacaagaaccggggagattacagacaccacatggtggacgctttttgcacctctctgatcagccccaaggttctggacatcattaacatcatgcggaagcagttcaacaagaaaacagagaagtacaaggagtgcgagacaaagttaaacgactacatcaagaacgttaagaatgatttcatcaaacacttcgacaatgtgatcacatcccacgaggtggaaagcaaactgaagggcgagctggaagaagagacactgtacggccacgagaagatcaagctggacgatggcagcatcataaccaagctgttccagcacaagccttacgaagaggtgattagcaagtataacagccctgaggaagtgctgaaggcccacgacaacctggaaatcagcctgccaaagggcctgaaaaagtacctggaaaacaacaacaaactgcccgacatgttccagggctggaaacgcatcaagaagtactacaacaacatcgatgagaacaacttcaacatcaacatctatagagccatccacaacgaaaaggagaaggtgatcgcctacaagaagacacaggagaatgcttacatcatcgtgtacaacgatttcaagaacgagacgatcagcaagatgaacgaaatcagcaacaaacctaagttcaacaacgtgttctgcaagctgtacaagggcgacctgatccaggattctgagaacaacatctacaagatataccagctgctgagcgacaagagaatcgccctgcaccccgtgaacatccagcctatcaaaaccaagcgcaagagcgtgaaactgatctttgataaggagaagatgtacaagatcaaggtgaacatcctgggtcacatcatc

SEQ ID NO: 16 - DNA, 36 bp, synthetic construct
  source 1..36: mol_type = other DNA
ggtaccgccaccatgccgaaaaagaagcgaaaggtc

SEQ ID NO: 17 - DNA, 54 bp, synthetic construct
  source 1..54: mol_type = other DNA
aaaaggccggcggccacgaaaaaggccggccaggcaaaaaagaaaaagtctaga

SEQ ID NO: 18 - DNA, 3042 bp, synthetic construct
  source 1..3042: mol_type = other DNA
atgccgaaaaagaagcgaaaggtcaccaaaaaagtgctgagcattgatcctggcgtgacctccatcggatggactctcacagagcagaacgagaagggccacctgacaaagttcatcgatggcggaagcagaatcttcaacagcgtgaaggaggccaaatctggcaccttcaagaatgagaagcggagagccaaaagaaccacccggagaaacaagtacagatctaacagaagaatggccaagctggagaactacctgatcaagaacgatttcctctctaataaaatcagcagcctgtccgaccacaccggcctggtgcagcaaatcatcggcaatccttaccacctgagaaagaaagccctttatgaacccctgaccaatgaagagctggcatgggccatcatccacctggccaagagacgcggcttcctgagctccagcaagagtctgaccccagaggagaagaaagaacaggctagagccgacgagttggctacactgatgaagaaggaaaagtgcaagaccctgggagagtacttcagcaacctgtacgacaagggtgagaagatcagaggcgaaaagctgaagcggcagctgatccaggacgagctggaactgattctgaataagcaaatggaaacaaatagcctgatcacctacaagttcgtgaatgatatcaataccatcatcttcaaccagagacctctgaagacccagaaaaggattagcctgtgtaaattcgagtcttttggaaagatcaagaagcacacagccgccaagctgcaccctctgagccagcagtttatcctgtggggcttcattaataatctgaaatataacgacaacagcggcggcatgcaggagctaaccctggaacagaaaaacgtggtgttcgacctgctttggaccaacaaggaagtgacctttaagaagatcatcaaagaactgaagctgacccctgaaacaacctttaacttccagaaaggcgaagatgacaaagtcaagggcaaccagctgctgaactacttcaaagccaaaacaaagacctggttcaacagcctgtctgaacagcagaagatcgatctgatacaggacctgtctacaatcaacgacctgacaggcttcgccctgaagaagcggatctataaccactggaccaaggatgaagagatcatcgagaacctgctgctgacctctgataagctgccacagggctacaccagcctttctctgaaggccaccaagaagatcctgcctttcctgaaagctggcaacaagtactacgaggccgagaagaaggcctatcctaacttcaccatcaacaccaagaaggttaacaaattgccccccgtggaaggcatcagcaacaccgtggtgctgaagagctgcagccaggtgcggcacctggtgaacgccattgtggacaagtacggcgagatcgacatcatcaagattgagctggctagagacctgagcaaaagcaagaaacaaatctcggaaactaatatcctgaattccaagaacaagtccctgaacgacgaggctatcagctacctgcacaagaacaacatcgacgtgaatcacgacaacatcaccaagtacaagctgtggaaggaaagcgaatctagcgacaagcaacacagaagctgctaccccgagcaggatagcgacggcaactggtttttccccacaatcaacctgaatgatctatatggcgccaacgccatctacgagatcgagcacatcatccctaagtccatcagcggcgacgatagcttcgccaacaaggctctctgcaaacacaaaaccaatgcccagaagggaaataaaaccccatacgactactactttcagaaaggaggacaggagctgatcgatatgatcgccaaaacagcctacagccagttcggaaaatggaagggcaagaagttcgtgacaagtaccgagaaatacctggacgaaaatgacatccagaagcgctacctcaatgacaccagatacctggccgtcttcctgaaagagtacctgcagcctgtgtgtaaggacaagatcgtggtgtccaaggggggttttaccgccatcattagacagagcctgaacctgaacatcctgctgggcaacgaattcaacaagaatagaggcgactacagacaccacatggtcgacgccttttgcaccagcctgatcagccctaaggtgctggacatcatcaacatcatgagaaaacagttcaacaaaaagacagaaaagtacaaggagtgcgagacaaagctgaacgattacattaagaacgtgaagaacgacttcatcaagcatttcgacaacgtgatcaccagccacgaggtggaatccaagctgaagggcgagctggaggaagaaacactgtacggccacgagaagataaagctggatgacggcagcatcatcacgaagctgttccaacacaagccatacgaggaagttatcagcaagtacaactcgcctgaggaagtcctgaaggcccacgataacctggagatcagcctgccgaagggcctgaaaaagtacctggaaaacaacaacaagctgcccgacatgttccagggctggaaacggatcaagaagtactacaacaacatcgacgagaacaacttcaacatcaacatctatcgggcgatccataacgagaaagagaaggtgatcgcctacaagaaaacacaggagaacgcctacatcatcgtgtacaacgacttcaagaacgagacaatctctaagatgaacgaaatcagcaacaagcctaagtttaacaatgtgttttgtaagctgtacaagggagatctgatccaagacagcgagaacaacatctacaagatataccagctgctgagcgacaagcgtatcgctctgcatcctgtgaacatccagcctatcaagaccaagcggaagagcgtgaagctcatcttcgataaggagaagatgtacaagatcaaggtgaacatcctgggccacatcatcaaaaggccggcggccacgaaaaaggccggccaggcaaaaaagaaaaag

SEQ ID NO: 19 - DNA, 3054 bp, synthetic construct
  source 1..3054: mol_type = other DNA
atgaaaatagaagagacaaaaaaggtactatcgatcgacccgggtgttacctccatcggctggaccttgaccgaacaaaacgagaagggtcacctgacgaagttcatcgacggcggcagccgtatcttcaactccgtgaaagaggcgaagagcggcacctttaaaaacgaaaagcgccgcgcgaagcgcaccacccgtcgtaataaataccgcagcaaccgtcgtatggcaaagctggaaaactatctgattaaaaacgactttttatccaacaaaatcagcagcctgagcgaccacacgggactggtccagcaaatcattggcaatccgtatcatctgcgtaaaaaggctctgtatgaaccgctgaccaacgaagagttggcctgggcaattatccacctggcgaagcgcagaggcttcctatcaagcagcaagagcttgactccagaagagaaaaaggagcaggcacgtgcggatgagttagcaaccctgatgaaaaaagagaagtgcaaaactctgggtgaatacttcagcaacttgtacgataaaggcgagaagatccgcggtgaaaagctgaaacgccagctgattcaagacgagctggaattgattctgaataagcaaatggaaaccaactctctaatcacctataaattcgtcaatgacatcaacaccattatttttaaccagcgtccgctgaagacccagaaacgcatctctctgtgtaaatttgaatccttcggtaaaatcaaaaaacacaccgctgccaagctgcacccgctgtcccagcagttcattctttggggttttatcaataacttgaaatacaatgacaactccggtggcatgcaagagctgactctggaacaaaaaaacgttgttttcgacttgctgtggacgaataaggaggtgacctttaagaagattatcaaggagctgaagttgaccccggaaacaaccttcaacttccaaaagggcgaagatgataaagtaaaaggaaaccagctgctgaattatttcaaagcgaagaccaaaacctggttcaacagtctgtccgagcaacaaaagattgacctgatccaggaccttagcaccattaacgacctgacgggtttcgccctaaagaaacgcatttataaccattggactaaggatgaagagataatcgaaaatctcctgctgacctcagacaagctgccgcagggctatacctctttgtctctgaaggcgaccaagaaaatcctgccgtttctcaaggcgggtaacaagtattacgaggctgaaaaaaaggcgtacccaaattttaccatcaacactaaaaaagttaacaaactgcctccggtagaaggtattagcaataccgttgttctgaagagctgcagccaggttcgtcacctggtcaacgcaattgttgataaatacggcgaaatcgacatcatcaaaattgagctcgcgcgtgatttgtcgaaaagcaaaaaacagatttctgagacgaatatccttaacagcaagaacaaaagcttgaacgacgaggcgatttcctatctgcacaaaaataacattgatgttaatcatgataacatcaccaagtacaagctgtggaaagaatcggaatcttctgataagcagcatcgtagctgttatccggagcaagattccgacggtaactggttttttccgaccatcaatctgaatgatctgtacggcgcaaatgccatctatgaaatcgagcacattattccgaagagcattagtggtgatgactcgttcgcaaataaagcgctttgcaagcacaagacgaatgcgcagaaaggcaacaaaactccgtatgattactacttccagaaaggtggccaggaactgattgacatgattgcgaagacggcttacagccagttcggtaaatggaagggcaaaaagttcgtgacctccaccgagaaatacctggatgaaaatgacattcaaaaacgttacttgaatgatacccgttatctggctgtgtttctgaaagagtatctgcagccggtgtgcaaggacaaaatcgtggtgagcaaaggcggtttcaccgcaattatccgccaaagcctcaacctgaatatactacttggtaacgaatttaataaaaatcgtggtgactaccgtcatcatatggttgacgcgttttgtaccagcctgattagcccgaaagtgctggatatcatcaacattatgcgtaaacaatttaacaaaaagacggaaaagtataaggagtgcgaaaccaagctcaacgactacatcaaaaacgtgaaaaacgattttatcaagcactttgacaacgttattaccagccatgaggtcgaaagcaagctgaaaggtgaattggaagaggagaccctgtacggtcacgaaaagattaaactcgacgacggctcgataatcacaaagttatttcagcacaaaccgtacgaggaggttattagcaaatacaactccccggaagaagtgctcaaggcgcatgacaacctggagatcagcttgccgaaaggcctgaagaaatacttggagaacaataacaagctcccagatatgtttcaaggttggaaacggattaaaaagtactacaataacatcgacgagaacaatttcaacatcaacatttaccgtgcgatccacaacgagaaagagaaggtgatcgcgtacaaaaaaacacaagaaaacgcttatattatcgtttataacgacttcaagaacgagaccatcagcaagatgaatgagatctccaacaaaccgaaattcaacaacgtgttctgcaagctgtataagggtgatttaatacaggattcggagaacaacatctacaaaatctatcagttgctgagcgataaacgtatagcgctgcatccggtcaacattcaaccgattaaaacgaaacgtaaatctgttaaactaatcttcgataaggagaagatgtataagatcaaggtgaacattctgggtcatattatctctcgtgctgatccgaagaaaaagaggaaggtggcggccgccctcgagcaccaccaccaccaccactga

SEQ ID NO: 20 - DNA, 158 bp, synthetic construct
  source 1..158: mol_type = other DNA
aagctaatacgactcactataggcggcaagatgagaatgactgattgtaattagttaacgaaagttaactagtgtattacaataagacaacattgttgtcgtaagttttaaactataaatagtctattgaaactcgatttcaataggcttttttcttt

SEQ ID NO: 21 - DNA, 135 bp, synthetic construct
  source 1..135: mol_type = other DNA
aagctaatacgactcactataggctaccataggcaccacgaggtttaagagctatgctggaaacagcatagcaagtttaaataaggctagtccgttatcaacttgaaaaagtggcaccgagtcggtgcttttttt

SEQ ID NO: 22 - DNA, 52 bp, Caenorhabditis elegans
  source 1..52: mol_type = genomic DNA
cttgaacttcaatacggcaagatgagaatgactggaaaccgtaccgctcgtg

SEQ ID NO: 23 - DNA, 48 bp, Caenorhabditis elegans
  source 1..48: mol_type = genomic DNA
cttgaacttcaatacggcaagatgagaatgaaaaccgtaccgctcgtg

SEQ ID NO: 24 - DNA, 47 bp, Caenorhabditis elegans
  source 1..47: mol_type = genomic DNA
cttgaacttcaatacggcaagatgagaatgaaaccgtaccgctcgtg

SEQ ID NO: 25 - DNA, 48 bp, Caenorhabditis elegans
  source 1..48: mol_type = genomic DNA
cttgaacttcaatacggcaagatgagaatggaaaccgtaccgctcgtg

SEQ ID NO: 26 - DNA, 47 bp, Caenorhabditis elegans
  source 1..47: mol_type = genomic DNA
cttgaacttcaatacggcaagatgaactggaaaccgtaccgctcgtg

SEQ ID NO: 27 - DNA, 44 bp, Caenorhabditis elegans
  source 1..44: mol_type = genomic DNA
cttgaacttcaatacggcaagatgagaataccgtaccgctcgtg

SEQ ID NO: 28 - DNA, 35 bp, Caenorhabditis elegans
  source 1..35: mol_type = genomic DNA
cttgaacttcaatacggaaaaccgtaccgctcgtg

SEQ ID NO: 29 - DNA, 29 bp, Caenorhabditis elegans
  source 1..29: mol_type = genomic DNA
cttgaacttcaaaaaccgtaccgctcgtg

SEQ ID NO: 30 - DNA, 53 bp, Caenorhabditis elegans
  source 1..53: mol_type = genomic DNA
cttgaacttcaatacggaaaccgtaccgcatactggaaaccgtaccgctcgtg